European Patent Specification EP 4 204 097 B1, published April 15, 2026. Title: Methods Of Treating Cancer. Applicant: Institute For Cancer Research d/b/a The Research Institute Of Fox Chase Cancer Center Bellacosa, Alfonso Yen, Timothy J. Karanicolas, John Cory, Michael Parry, Chris Prasad, Rahul. The sequence listing filed with the application follows.

SEQUENCE LISTING (2 sequences)

SEQ ID NO: 1 - DNA, 43 bp, artificial sequence
  Synthetic sequence; hairpin G:U mismatched substrate
ccactugtgaattgacagcccatgtgcatcaattcacgagtgg

SEQ ID NO: 2 - DNA, 5 bp, artificial sequence
  Synthetic sequence; internal standard
ttttt